European Patent Specification EP 3 413 933 B1, published April 8, 2026. Title: DENDRIMER-BIOADHESIVE POLYMER HYDROGEL NANOGEL AND USE THEREOF. Applicant: Johns Hopkins Tecnology Ventures. The sequence listing filed with the application follows.

SEQUENCE LISTING (12 sequences)

SEQ ID NO: 1 - DNA, 18 bp, Artificial Sequence
  synthetic sequence
gcaagagagaggccctca

SEQ ID NO: 2 - DNA, 20 bp, Artificial Sequence
  synthetic sequence
tgtgagggagatgctcagtg

SEQ ID NO: 3 - DNA, 19 bp, Artificial Sequence
  synthetic sequence
tcagttccatggcccagac

SEQ ID NO: 4 - DNA, 24 bp, Artificial Sequence
  synthetic sequence
gttgtctttgagatccatgccatt

SEQ ID NO: 5 - DNA, 21 bp, Artificial Sequence
  synthetic sequence
cacctctcaagcagagcacag

SEQ ID NO: 6 - DNA, 21 bp, Artificial Sequence
  synthetic sequence
gggttccatggtgaagtcaac

SEQ ID NO: 7 - DNA, 24 bp, Artificial Sequence
  synthetic sequence
aaagagttgtgcaatggcaattct

SEQ ID NO: 8 - DNA, 24 bp, Artificial Sequence
  synthetic sequence
cagtgcatcatcgctgttcataca

SEQ ID NO: 9 - DNA, 24 bp, Artificial Sequence
  synthetic sequence
ctatgcaggtctctgtcacgcttc

SEQ ID NO: 10 - DNA, 20 bp, Artificial Sequence
  synthetic sequence
cagccgactcattgggatca

SEQ ID NO: 11 - DNA, 20 bp, Artificial Sequence
  synthetic sequence
ggctttactgctgtacctcc

SEQ ID NO: 12 - DNA, 19 bp, Artificial Sequence
  synthetic sequence
caaatgctttctccgctct